European Patent Application EP 4 169 525 A1, published April 26, 2023. Title: Factor VIII Chimeric and Hybrid Polypeptides, and Methods of Use Thereof. Applicant: Bioverative Therapeutics. The sequence listing filed with the application follows.

SEQUENCE LISTING (16 sequences)

SEQ ID NO: 1 - DNA, 5052 bp, Artificial Sequence
  B-Domain Deleted FVIIIFc Chain
  misc_feature (1)..(57): FVIII signal
  misc_feature (4372)..(5052): Fc region
atgcaaatagagctctccacctgcttctttctgtgccttttgcgattctgctttagtgccaccagaagatactacctgggtgcagtggaactgtcatgggactatatgcaaagtgatctcggtgagctgcctgtggacgcaagatttcctcctagagtgccaaaatcttttccattcaacacctcagtcgtgtacaaaaagactctgtttgtagaattcacggatcaccttttcaacatcgctaagccaaggccaccctggatgggtctgctaggtcctaccatccaggctgaggtttatgatacagtggtcattacacttaagaacatggcttcccatcctgtcagtcttcatgctgttggtgtatcctactggaaagcttctgagggagctgaatatgatgatcagaccagtcaaagggagaaagaagatgataaagtcttccctggtggaagccatacatatgtctggcaggtcctgaaagagaatggtccaatggcctctgacccactgtgccttacctactcatatctttctcatgtggacctggtaaaagacttgaattcaggcctcattggagccctactagtatgtagagaagggagtctggccaaggaaaagacacagaccttgcacaaatttatactactttttgctgtatttgatgaagggaaaagttggcactcagaaacaaagaactccttgatgcaggatagggatgctgcatctgctcgggcctggcctaaaatgcacacagtcaatggttatgtaaacaggtctctgccaggtctgattggatgccacaggaaatcagtctattggcatgtgattggaatgggcaccactcctgaagtgcactcaatattcctcgaaggtcacacatttcttgtgaggaaccatcgccaggcgtccttggaaatctcgccaataactttccttactgctcaaacactcttgatggaccttggacagtttctactgttttgtcatatctcttcccaccaacatgatggcatggaagcttatgtcaaagtagacagctgtccagaggaaccccaactacgaatgaaaaataatgaagaagcggaagactatgatgatgatcttactgattctgaaatggatgtggtcaggtttgatgatgacaactctccttcctttatccaaattcgctcagttgccaagaagcatcctaaaacttgggtacattacattgctgctgaagaggaggactgggactatgctcccttagtcctcgcccccgatgacagaagttataaaagtcaatatttgaacaatggccctcagcggattggtaggaagtacaaaaaagtccgatttatggcatacacagatgaaacctttaagactcgtgaagctattcagcatgaatcaggaatcttgggacctttactttatggggaagttggagacacactgttgattatatttaagaatcaagcaagcagaccatataacatctaccctcacggaatcactgatgtccgtcctttgtattcaaggagattaccaaaaggtgtaaaacatttgaaggattttccaattctgccaggagaaatattcaaatataaatggacagtgactgtagaagatgggccaactaaatcagatcctcggtgcctgacccgctattactctagtttcgttaatatggagagagatctagcttcaggactcattggccctctcctcatctgctacaaagaatctgtagatcaaagaggaaaccagataatgtcagacaagaggaatgtcatcctgttttctgtatttgatgagaaccgaagctggtacctcacagagaatatacaacgctttctccccaatccagctggagtgcagcttgaggatccagagttccaagcctccaacatcatgcacagcatcaatggctatgtttttgatagtttgcagttgtcagtttgtttgcatgaggtggcatactggtacattctaagcattggagcacagactgacttcctttctgtcttcttctctggatataccttcaaacacaaaatggtctatgaagacacactcaccctattcccattctcaggagaaactgtcttcatgtcgatggaaaacccaggtctatggattctggggtgccacaactcagactttcggaacagaggcatgaccgccttactgaaggtttctagttgtgacaagaacactggtgattattacgaggacagttatgaagatatttcagcatacttgctgagtaaaaacaatgccattgaaccaagaagcttctctcaaaacccaccagtcttgaaacgccatcaacgggaaataactcgtactactcttcagtcagatcaagaggaaattgactatgatgataccatatcagttgaaatgaagaaggaagattttgacatttatgatgaggatgaaaatcagagcccccgcagctttcaaaagaaaacacgacactattttattgctgcagtggagaggctctgggattatgggatgagtagctccccacatgttctaagaaacagggctcagagtggcagtgtccctcagttcaagaaagttgttttccaggaatttactgatggctcctttactcagcccttataccgtggagaactaaatgaacatttgggactcctggggccatatataagagcagaagttgaagataatatcatggtaactttcagaaatcaggcctctcgtccctattccttctattctagccttatttcttatgaggaagatcagaggcaaggagcagaacctagaaaaaactttgtcaagcctaatgaaaccaaaacttacttttggaaagtgcaacatcatatggcacccactaaagatgagtttgactgcaaagcctgggcttatttctctgatgttgacctggaaaaagatgtgcactcaggcctgattggaccccttctggtctgccacactaacacactgaaccctgctcatgggagacaagtgacagtacaggaatttgctctgtttttcaccatctttgatgagaccaaaagctggtacttcactgaaaatatggaaagaaactgcagggctccctgcaatatccagatggaagatcccacttttaaagagaattatcgcttccatgcaatcaatggctacataatggatacactacctggcttagtaatggctcaggatcaaaggattcgatggtatctgctcagcatgggcagcaatgaaaacatccattctattcatttcagtggacatgtgttcactgtacgaaaaaaagaggagtataaaatggcactgtacaatctctatccaggtgtttttgagacagtggaaatgttaccatccaaagctggaatttggcgggtggaatgccttattggcgagcatctacatgctgggatgagcacactttttctggtgtacagcaataagtgtcagactcccctgggaatggcttctggacacattagagattttcagattacagcttcaggacaatatggacagtgggccccaaagctggccagacttcattattccggatcaatcaatgcctggagcaccaaggagcccttttcttggatcaaggtggatctgttggcaccaatgattattcacggcatcaagacccagggtgcccgtcagaagttctccagcctctacatctctcagtttatcatcatgtatagtcttgatgggaagaagtggcagacttatcgaggaaattccactggaaccttaatggtcttctttggcaatgtggattcatctgggataaaacacaatatttttaaccctccaattattgctcgatacatccgtttgcacccaactcattatagcattcgcagcactcttcgcatggagttgatgggctgtgatttaaatagttgcagcatgccattgggaatggagagtaaagcaatatcagatgcacagattactgcttcatcctactttaccaatatgtttgccacctggtctccttcaaaagctcgacttcacctccaagggaggagtaatgcctggagacctcaggtgaataatccaaaagagtggctgcaagtggacttccagaagacaatgaaagtcacaggagtaactactcagggagtaaaatctctgcttaccagcatgtatgtgaaggagttcctcatctccagcagtcaagatggccatcagtggactctcttttttcagaatggcaaagtaaaggtttttcagggaaatcaagactccttcacacctgtggtgaactctctagacccaccgttactgactcgctaccttcgaattcacccccagagttgggtgcaccagattgccctgaggatggaggttctgggctgcgaggcacaggacctctacgacaaaactcacacatgcccaccgtgcccagctccagaactcctgggcggaccgtcagtcttcctcttccccccaaaacccaaggacaccctcatgatctcccggacccctgaggtcacatgcgtggtggtggacgtgagccacgaagaccctgaggtcaagttcaactggtacgtggacggcgtggaggtgcataatgccaagacaaagccgcgggaggagcagtacaacagcacgtaccgtgtggtcagcgtcctcaccgtcctgcaccaggactggctgaatggcaaggagtacaagtgcaaggtctccaacaaagccctcccagcccccatcgagaaaaccatctccaaagccaaagggcagccccgagaaccacaggtgtacaccctgcccccatcccgggatgagctgaccaagaaccaggtcagcctgacctgcctggtcaaaggcttctatcccagcgacatcgccgtggagtgggagagcaatgggcagccggagaacaactacaagaccacgcctcccgtgttggactccgacggctccttcttcctctacagcaagctcaccgtggacaagagcaggtggcagcaggggaacgtcttctcatgctccgtgatgcatgaggctctgcacaaccactacacgcagaagagcctctccctgtctccgggtaaa

SEQ ID NO: 2 - protein, 1684 aa, Artificial Sequence
  B domain deleted FVIII-Fc chain
  MISC_FEATURE (1)..(19): Signal
  MISC_FEATURE (20)..(753): Heavy chain (HC)
  MISC_FEATURE (760)..(773): B domain
  MISC_FEATURE (1457)..(1684): Fc region
MQIELSTCFFLCLLRFCFSATRRYYLGAVELSWDYMQSDLGELPVDARFPPRVPKSFPFNTSVVYKKTLFVEFTDHLFNIAKPRPPWMGLLGPTIQAEVYDTVVITLKNMASHPVSLHAVGVSYWKASEGAEYDDQTSQREKEDDKVFPGGSHTYVWQVLKENGPMASDPLCLTYSYLSHVDLVKDLNSGLIGALLVCREGSLAKEKTQTLHKFILLFAVFDEGKSWHSETKNSLMQDRDAASARAWPKMHTVNGYVNRSLPGLIGCHRKSVYWHVIGMGTTPEVHSIFLEGHTFLVRNHRQASLEISPITFLTAQTLLMDLGQFLLFCHISSHQHDGMEAYVKVDSCPEEPQLRMKNNEEAEDYDDDLTDSEMDVVRFDDDNSPSFIQIRSVAKKHPKTWVHYIAAEEEDWDYAPLVLAPDDRSYKSQYLNNGPQRIGRKYKKVRFMAYTDETFKTREAIQHESGILGPLLYGEVGDTLLIIFKNQASRPYNIYPHGITDVRPLYSRRLPKGVKHLKDFPILPGEIFKYKWTVTVEDGPTKSDPRCLTRYYSSFVNMERDLASGLIGPLLICYKESVDQRGNQIMSDKRNVILFSVFDENRSWYLTENIQRFLPNPAGVQLEDPEFQASNIMHSINGYVFDSLQLSVCLHEVAYWYILSIGAQTDFLSVFFSGYTFKHKMVYEDTLTLFPFSGETVFMSMENPGLWILGCHNSDFRNRGMTALLKVSSCDKNTGDYYEDSYEDISAYLLSKNNAIEPRSFSQNPPVLKRHQREITRTTLQSDQEEIDYDDTISVEMKKEDFDIYDEDENQSPRSFQKKTRHYFIAAVERLWDYGMSSSPHVLRNRAQSGSVPQFKKVVFQEFTDGSFTQPLYRGELNEHLGLLGPYIRAEVEDNIMVTFRNQASRPYSFYSSLISYEEDQRQGAEPRKNFVKPNETKTYFWKVQHHMAPTKDEFDCKAWAYFSDVDLEKDVHSGLIGPLLVCHTNTLNPAHGRQVTVQEFALFFTIFDETKSWYFTENMERNCRAPCNIQMEDPTFKENYRFHAINGYIMDTLPGLVMAQDQRIRWYLLSMGSNENIHSIHFSGHVFTVRKKEEYKMALYNLYPGVFETVEMLPSKAGIWRVECLIGEHLHAGMSTLFLVYSNKCQTPLGMASGHIRDFQITASGQYGQWAPKLARLHYSGSINAWSTKEPFSWIKVDLLAPMIIHGIKTQGARQKFSSLYISQFIIMYSLDGKKWQTYRGNSTGTLMVFFGNVDSSGIKHNIFNPPIIARYIRLHPTHYSIRSTLRMELMGCDLNSCSMPLGMESKAISDAQITASSYFTNMFATWSPSKARLHLQGRSNAWRPQVNNPKEWLQVDFQKTMKVTGVTTQGVKSLLTSMYVKEFLISSSQDGHQWTLFFQNGKVKVFQGNQDSFTPVVNSLDPPLLTRYLRIHPQSWVHQIALRMEVLGCEAQDLYDKTHTCPPCPAPELLGGPSVFLFPPKPKDTLMISRTPEVTCVVVDVSHEDPEVKFNWYVDGVEVHNAKTKPREEQYNSTYRVVSVLTVLHQDWLNGKEYKCKVSNKALPAPIEKTISKAKGQPREPQVYTLPPSRDELTKNQVSLTCLVKGFYPSDIAVEWESNGQPENNYKTTPPVLDSDGSFFLYSKLTVDKSRWQQGNVFSCSVMHEALHNHYTQKSLSLSPGK

SEQ ID NO: 3 - DNA, 741 bp, Artificial Sequence
  Fc region
  misc_signal (1)..(60): Mouse Ig kappa signal
atggagacagacacactcctgctatgggtactgctgctctgggttccaggttccactggtgacaaaactcacacatgcccaccgtgcccagcacctgaactcctgggaggaccgtcagtcttcctcttccccccaaaacccaaggacaccctcatgatctcccggacccctgaggtcacatgcgtggtggtggacgtgagccacgaagaccctgaggtcaagttcaactggtacgtggacggcgtggaggtgcataatgccaagacaaagccgcgggaggagcagtacaacagcacgtaccgtgtggtcagcgtcctcaccgtcctgcaccaggactggctgaatggcaaggagtacaagtgcaaggtctccaacaaagccctcccagcccccatcgagaaaaccatctccaaagccaaagggcagccccgagaaccacaggtgtacaccctgcccccatcccgcgatgagctgaccaagaaccaggtcagcctgacctgcctggtcaaaggcttctatcccagcgacatcgccgtggagtgggagagcaatgggcagccggagaacaactacaagaccacgcctcccgtgttggactccgacggctccttcttcctctacagcaagctcaccgtggacaagagcaggtggcagcaggggaacgtcttctcatgctccgtgatgcatgaggctctgcacaaccactacacgcagaagagcctctccctgtctccgggtaaa

SEQ ID NO: 4 - protein, 247 aa, Artificial Sequence
  Fc chain
  MISC_FEATURE (1)..(20): heterologous signal from Mouse Ig kappa chain
METDTLLLWVLLLWVPGSTGDKTHTCPPCPAPELLGGPSVFLFPPKPKDTLMISRTPEVTCVVVDVSHEDPEVKFNWYVDGVEVHNAKTKPREEQYNSTYRVVSVLTVLHQDWLNGKEYKCKVSNKALPAPIEKTISKAKGQPREPQVYTLPPSRDELTKNQVSLTCLVKGFYPSDIAVEWESNGQPENNYKTTPPVLDSDGSFFLYSKLTVDKSRWQQGNVFSCSVMHEALHNHYTQKSLSLSPGK

SEQ ID NO: 5 - DNA, 7734 bp, Artificial Sequence
  Full length FVIIIFc
  misc_signal (1)..(57): FVIII signal
  misc_feature (7054)..(7734): Fc region
atgcaaatagagctctccacctgcttctttctgtgccttttgcgattctgctttagtgccaccagaagatactacctgggtgcagtggaactgtcatgggactatatgcaaagtgatctcggtgagctgcctgtggacgcaagatttcctcctagagtgccaaaatcttttccattcaacacctcagtcgtgtacaaaaagactctgtttgtagaattcacggatcaccttttcaacatcgctaagccaaggccaccctggatgggtctgctaggtcctaccatccaggctgaggtttatgatacagtggtcattacacttaagaacatggcttcccatcctgtcagtcttcatgctgttggtgtatcctactggaaagcttctgagggagctgaatatgatgatcagaccagtcaaagggagaaagaagatgataaagtcttccctggtggaagccatacatatgtctggcaggtcctgaaagagaatggtccaatggcctctgacccactgtgccttacctactcatatctttctcatgtggacctggtaaaagacttgaattcaggcctcattggagccctactagtatgtagagaagggagtctggccaaggaaaagacacagaccttgcacaaatttatactactttttgctgtatttgatgaagggaaaagttggcactcagaaacaaagaactccttgatgcaggatagggatgctgcatctgctcgggcctggcctaaaatgcacacagtcaatggttatgtaaacaggtctctgccaggtctgattggatgccacaggaaatcagtctattggcatgtgattggaatgggcaccactcctgaagtgcactcaatattcctcgaaggtcacacatttcttgtgaggaaccatcgccaggcgtccttggaaatctcgccaataactttccttactgctcaaacactcttgatggaccttggacagtttctactgttttgtcatatctcttcccaccaacatgatggcatggaagcttatgtcaaagtagacagctgtccagaggaaccccaactacgaatgaaaaataatgaagaagcggaagactatgatgatgatcttactgattctgaaatggatgtggtcaggtttgatgatgacaactctccttcctttatccaaattcgctcagttgccaagaagcatcctaaaacttgggtacattacattgctgctgaagaggaggactgggactatgctcccttagtcctcgcccccgatgacagaagttataaaagtcaatatttgaacaatggccctcagcggattggtaggaagtacaaaaaagtccgatttatggcatacacagatgaaacctttaagactcgtgaagctattcagcatgaatcaggaatcttgggacctttactttatggggaagttggagacacactgttgattatatttaagaatcaagcaagcagaccatataacatctaccctcacggaatcactgatgtccgtcctttgtattcaaggagattaccaaaaggtgtaaaacatttgaaggattttccaattctgccaggagaaatattcaaatataaatggacagtgactgtagaagatgggccaactaaatcagatcctcggtgcctgacccgctattactctagtttcgttaatatggagagagatctagcttcaggactcattggccctctcctcatctgctacaaagaatctgtagatcaaagaggaaaccagataatgtcagacaagaggaatgtcatcctgttttctgtatttgatgagaaccgaagctggtacctcacagagaatatacaacgctttctccccaatccagctggagtgcagcttgaggatccagagttccaagcctccaacatcatgcacagcatcaatggctatgtttttgatagtttgcagttgtcagtttgtttgcatgaggtggcatactggtacattctaagcattggagcacagactgacttcctttctgtcttcttctctggatataccttcaaacacaaaatggtctatgaagacacactcaccctattcccattctcaggagaaactgtcttcatgtcgatggaaaacccaggtctatggattctggggtgccacaactcagactttcggaacagaggcatgaccgccttactgaaggtttctagttgtgacaagaacactggtgattattacgaggacagttatgaagatatttcagcatacttgctgagtaaaaacaatgccattgaaccaagaagcttctcccagaattcaagacaccctagcactaggcaaaagcaatttaatgccaccacaattccagaaaatgacatagagaagactgacccttggtttgcacacagaacacctatgcctaaaatacaaaatgtctcctctagtgatttgttgatgctcttgcgacagagtcctactccacatgggctatccttatctgatctccaagaagccaaatatgagactttttctgatgatccatcacctggagcaatagacagtaataacagcctgtctgaaatgacacacttcaggccacagctccatcacagtggggacatggtatttacccctgagtcaggcctccaattaagattaaatgagaaactggggacaactgcagcaacagagttgaagaaacttgatttcaaagtttctagtacatcaaataatctgatttcaacaattccatcagacaatttggcagcaggtactgataatacaagttccttaggacccccaagtatgccagttcattatgatagtcaattagataccactctatttggcaaaaagtcatctccccttactgagtctggtggacctctgagcttgagtgaagaaaataatgattcaaagttgttagaatcaggtttaatgaatagccaagaaagttcatggggaaaaaatgtatcgtcaacagagagtggtaggttatttaaagggaaaagagctcatggacctgctttgttgactaaagataatgccttattcaaagttagcatctctttgttaaagacaaacaaaacttccaataattcagcaactaatagaaagactcacattgatggcccatcattattaattgagaatagtccatcagtctggcaaaatatattagaaagtgacactgagtttaaaaaagtgacacctttgattcatgacagaatgcttatggacaaaaatgctacagctttgaggctaaatcatatgtcaaataaaactacttcatcaaaaaacatggaaatggtccaacagaaaaaagagggccccattccaccagatgcacaaaatccagatatgtcgttctttaagatgctattcttgccagaatcagcaaggtggatacaaaggactcatggaaagaactctctgaactctgggcaaggccccagtccaaagcaattagtatccttaggaccagaaaaatctgtggaaggtcagaatttcttgtctgagaaaaacaaagtggtagtaggaaagggtgaatttacaaaggacgtaggactcaaagagatggtttttccaagcagcagaaacctatttcttactaacttggataatttacatgaaaataatacacacaatcaagaaaaaaaaattcaggaagaaatagaaaagaaggaaacattaatccaagagaatgtagttttgcctcagatacatacagtgactggcactaagaatttcatgaagaaccttttcttactgagcactaggcaaaatgtagaaggttcatatgacggggcatatgctccagtacttcaagattttaggtcattaaatgattcaacaaatagaacaaagaaacacacagctcatttctcaaaaaaaggggaggaagaaaacttggaaggcttgggaaatcaaaccaagcaaattgtagagaaatatgcatgcaccacaaggatatctcctaatacaagccagcagaattttgtcacgcaacgtagtaagagagctttgaaacaattcagactcccactagaagaaacagaacttgaaaaaaggataattgtggatgacacctcaacccagtggtccaaaaacatgaaacatttgaccccgagcaccctcacacagatagactacaatgagaaggagaaaggggccattactcagtctcccttatcagattgccttacgaggagtcatagcatccctcaagcaaatagatctccattacccattgcaaaggtatcatcatttccatctattagacctatatatctgaccagggtcctattccaagacaactcttctcatcttccagcagcatcttatagaaagaaagattctggggtccaagaaagcagtcatttcttacaaggagccaaaaaaaataacctttctttagccattctaaccttggagatgactggtgatcaaagagaggttggctccctggggacaagtgccacaaattcagtcacatacaagaaagttgagaacactgttctcccgaaaccagacttgcccaaaacatctggcaaagttgaattgcttccaaaagttcacatttatcagaaggacctattccctacggaaactagcaatgggtctcctggccatctggatctcgtggaagggagccttcttcagggaacagagggagcgattaagtggaatgaagcaaacagacctggaaaagttccctttctgagagtagcaacagaaagctctgcaaagactccctccaagctattggatcctcttgcttgggataaccactatggtactcagataccaaaagaagagtggaaatcccaagagaagtcaccagaaaaaacagcttttaagaaaaaggataccattttgtccctgaacgcttgtgaaagcaatcatgcaatagcagcaataaatgagggacaaaataagcccgaaatagaagtcacctgggcaaagcaaggtaggactgaaaggctgtgctctcaaaacccaccagtcttgaaacgccatcaacgggaaataactcgtactactcttcagtcagatcaagaggaaattgactatgatgataccatatcagttgaaatgaagaaggaagattttgacatttatgatgaggatgaaaatcagagcccccgcagctttcaaaagaaaacacgacactattttattgctgcagtggagaggctctgggattatgggatgagtagctccccacatgttctaagaaacagggctcagagtggcagtgtccctcagttcaagaaagttgttttccaggaatttactgatggctcctttactcagcccttataccgtggagaactaaatgaacatttgggactcctggggccatatataagagcagaagttgaagataatatcatggtaactttcagaaatcaggcctctcgtccctattccttctattctagccttatttcttatgaggaagatcagaggcaaggagcagaacctagaaaaaactttgtcaagcctaatgaaaccaaaacttacttttggaaagtgcaacatcatatggcacccactaaagatgagtttgactgcaaagcctgggcttatttctctgatgttgacctggaaaaagatgtgcactcaggcctgattggaccccttctggtctgccacactaacacactgaaccctgctcatgggagacaagtgacagtacaggaatttgctctgtttttcaccatctttgatgagaccaaaagctggtacttcactgaaaatatggaaagaaactgcagggctccctgcaatatccagatggaagatcccacttttaaagagaattatcgcttccatgcaatcaatggctacataatggatacactacctggcttagtaatggctcaggatcaaaggattcgatggtatctgctcagcatgggcagcaatgaaaacatccattctattcatttcagtggacatgtgttcactgtacgaaaaaaagaggagtataaaatggcactgtacaatctctatccaggtgtttttgagacagtggaaatgttaccatccaaagctggaatttggcgggtggaatgccttattggcgagcatctacatgctgggatgagcacactttttctggtgtacagcaataagtgtcagactcccctgggaatggcttctggacacattagagattttcagattacagcttcaggacaatatggacagtgggccccaaagctggccagacttcattattccggatcaatcaatgcctggagcaccaaggagcccttttcttggatcaaggtggatctgttggcaccaatgattattcacggcatcaagacccagggtgcccgtcagaagttctccagcctctacatctctcagtttatcatcatgtatagtcttgatgggaagaagtggcagacttatcgaggaaattccactggaaccttaatggtcttctttggcaatgtggattcatctgggataaaacacaatatttttaaccctccaattattgctcgatacatccgtttgcacccaactcattatagcattcgcagcactcttcgcatggagttgatgggctgtgatttaaatagttgcagcatgccattgggaatggagagtaaagcaatatcagatgcacagattactgcttcatcctactttaccaatatgtttgccacctggtctccttcaaaagctcgacttcacctccaagggaggagtaatgcctggagacctcaggtgaataatccaaaagagtggctgcaagtggacttccagaagacaatgaaagtcacaggagtaactactcagggagtaaaatctctgcttaccagcatgtatgtgaaggagttcctcatctccagcagtcaagatggccatcagtggactctcttttttcagaatggcaaagtaaaggtttttcagggaaatcaagactccttcacacctgtggtgaactctctagacccaccgttactgactcgctaccttcgaattcacccccagagttgggtgcaccagattgccctgaggatggaggttctgggctgcgaggcacaggacctctacgacaaaactcacacatgcccaccgtgcccagctccagaactcctgggcggaccgtcagtcttcctcttccccccaaaacccaaggacaccctcatgatctcccggacccctgaggtcacatgcgtggtggtggacgtgagccacgaagaccctgaggtcaagttcaactggtacgtggacggcgtggaggtgcataatgccaagacaaagccgcgggaggagcagtacaacagcacgtaccgtgtggtcagcgtcctcaccgtcctgcaccaggactggctgaatggcaaggagtacaagtgcaaggtctccaacaaagccctcccagcccccatcgagaaaaccatctccaaagccaaagggcagccccgagaaccacaggtgtacaccctgcccccatcccgggatgagctgaccaagaaccaggtcagcctgacctgcctggtcaaaggcttctatcccagcgacatcgccgtggagtgggagagcaatgggcagccggagaacaactacaagaccacgcctcccgtgttggactccgacggctccttcttcctctacagcaagctcaccgtggacaagagcaggtggcagcaggggaacgtcttctcatgctccgtgatgcatgaggctctgcacaaccactacacgcagaagagcctctccctgtctccgggtaaa

SEQ ID NO: 6 - protein, 2578 aa, Artificial Sequence
  Full length FVIIIFc chain
  MISC_FEATURE (1)..(19): FVIII signal
  MISC_FEATURE (20)..(759): HC
  MISC_FEATURE (760)..(1667): B domain
  MISC_FEATURE (2352)..(2578): Fc region
MQIELSTCFFLCLLRFCFSATRRYYLGAVELSWDYMQSDLGELPVDARFPPRVPKSFPFNTSVVYKKTLFVEFTDHLFNIAKPRPPWMGLLGPTIQAEVYDTVVITLKNMASHPVSLHAVGVSYWKASEGAEYDDQTSQREKEDDKVFPGGSHTYVWQVLKENGPMASDPLCLTYSYLSHVDLVKDLNSGLIGALLVCREGSLAKEKTQTLHKFILLFAVFDEGKSWHSETKNSLMQDRDAASARAWPKMHTVNGYVNRSLPGLIGCHRKSVYWHVIGMGTTPEVHSIFLEGHTFLVRNHRQASLEISPITFLTAQTLLMDLGQFLLFCHISSHQHDGMEAYVKVDSCPEEPQLRMKNNEEAEDYDDDLTDSEMDVVRFDDDNSPSFIQIRSVAKKHPKTWVHYIAAEEEDWDYAPLVLAPDDRSYKSQYLNNGPQRIGRKYKKVRFMAYTDETFKTREAIQHESGILGPLLYGEVGDTLLIIFKNQASRPYNIYPHGITDVRPLYSRRLPKGVKHLKDFPILPGEIFKYKWTVTVEDGPTKSDPRCLTRYYSSFVNMERDLASGLIGPLLICYKESVDQRGNQIMSDKRNVILFSVFDENRSWYLTENIQRFLPNPAGVQLEDPEFQASNIMHSINGYVFDSLQLSVCLHEVAYWYILSIGAQTDFLSVFFSGYTFKHKMVYEDTLTLFPFSGETVFMSMENPGLWILGCHNSDFRNRGMTALLKVSSCDKNTGDYYEDSYEDISAYLLSKNNAIEPRSFSQNSRHPSTRQKQFNATTIPENDIEKTDPWFAHRTPMPKIQNVSSSDLLMLLRQSPTPHGLSLSDLQEAKYETFSDDPSPGAIDSNNSLSEMTHFRPQLHHSGDMVFTPESGLQLRLNEKLGTTAATELKKLDFKVSSTSNNLISTIPSDNLAAGTDNTSSLGPPSMPVHYDSQLDTTLFGKKSSPLTESGGPLSLSEENNDSKLLESGLMNSQESSWGKNVSSTESGRLFKGKRAHGPALLTKDNALFKVSISLLKTNKTSNNSATNRKTHIDGPSLLIENSPSVWQNILESDTEFKKVTPLIHDRMLMDKNATALRLNHMSNKTTSSKNMEMVQQKKEGPIPPDAQNPDMSFFKMLFLPESARWIQRTHGKNSLNSGQGPSPKQLVSLGPEKSVEGQNFLSEKNKVVVGKGEFTKDVGLKEMVFPSSRNLFLTNLDNLHENNTHNQEKKIQEEIEKKETLIQENVVLPQIHTVTGTKNFMKNLFLLSTRQNVEGSYDGAYAPVLQDFRSLNDSTNRTKKHTAHFSKKGEEENLEGLGNQTKQIVEKYACTTRISPNTSQQNFVTQRSKRALKQFRLPLEETELEKRIIVDDTSTQWSKNMKHLTPSTLTQIDYNEKEKGAITQSPLSDCLTRSHSIPQANRSPLPIAKVSSFPSIRPIYLTRVLFQDNSSHLPAASYRKKDSGVQESSHFLQGAKKNNLSLAILTLEMTGDQREVGSLGTSATNSVTYKKVENTVLPKPDLPKTSGKVELLPKVHIYQKDLFPTETSNGSPGHLDLVEGSLLQGTEGAIKWNEANRPGKVPFLRVATESSAKTPSKLLDPLAWDNHYGTQIPKEEWKSQEKSPEKTAFKKKDTILSLNACESNHAIAAINEGQNKPEIEVTWAKQGRTERLCSQNPPVLKRHQREITRTTLQSDQEEIDYDDTISVEMKKEDFDIYDEDENQSPRSFQKKTRHYFIAAVERLWDYGMSSSPHVLRNRAQSGSVPQFKKVVFQEFTDGSFTQPLYRGELNEHLGLLGPYIRAEVEDNIMVTFRNQASRPYSFYSSLISYEEDQRQGAEPRKNFVKPNETKTYFWKVQHHMAPTKDEFDCKAWAYFSDVDLEKDVHSGLIGPLLVCHTNTLNPAHGRQVTVQEFALFFTIFDETKSWYFTENMERNCRAPCNIQMEDPTFKENYRFHAINGYIMDTLPGLVMAQDQRIRWYLLSMGSNENIHSIHFSGHVFTVRKKEEYKMALYNLYPGVFETVEMLPSKAGIWRVECLIGEHLHAGMSTLFLVYSNKCQTPLGMASGHIRDFQITASGQYGQWAPKLARLHYSGSINAWSTKEPFSWIKVDLLAPMIIHGIKTQGARQKFSSLYISQFIIMYSLDGKKWQTYRGNSTGTLMVFFGNVDSSGIKHNIFNPPIIARYIRLHPTHYSIRSTLRMELMGCDLNSCSMPLGMESKAISDAQITASSYFTNMFATWSPSKARLHLQGRSNAWRPQVNNPKEWLQVDFQKTMKVTGVTTQGVKSLLTSMYVKEFLISSSQDGHQWTLFFQNGKVKVFQGNQDSFTPVVNSLDPPLLTRYLRIHPQSWVHQIALRMEVLGCEAQDLYDKTHTCPPCPAPELLGGPSVFLFPPKPKDTLMISRTPEVTCVVVDVSHEDPEVKFNWYVDGVEVHNAKTKPREEQYNSTYRVVSVLTVLHQDWLNGKEYKCKVSNKALPAPIEKTISKAKGQPREPQVYTLPPSRDELTKNQVSLTCLVKGFYPSDIAVEWESNGQPENNYKTTPPVLDSDGSFFLYSKLTVDKSRWQQGNVFSCSVMHEALHNHYTQKSLSLSPGK

SEQ ID NO: 7 - protein, 11 aa, Artificial Sequence
  albumin-binding peptide
DICLPRWGCLW

SEQ ID NO: 8 - protein, 32 aa, Artificial Sequence
  CTP peptide
DPRFQDSSSSKAPPPSLPSPSRLPGPSDTPIL

SEQ ID NO: 9 - protein, 28 aa, Artificial Sequence
  CTP Petptide
SSSSKAPPPSLPSPSRLPGPSDTPILPQ

SEQ ID NO: 10 - protein, 20 aa, Artificial Sequence
  PAS peptide
ASPAAPAPASPAAPAPSAPA

SEQ ID NO: 11 - protein, 20 aa, Artificial Sequence
  PAS peptide
AAPASPAPAAPSAPAPAAPS

SEQ ID NO: 12 - protein, 20 aa, Artificial Sequence
  PAS peptide
APSSPSPSAPSSPSPASPSS

SEQ ID NO: 13 - protein, 19 aa, Artificial Sequence
  PAS peptide
APSSPSPSAPSSPSPASPS

SEQ ID NO: 14 - protein, 20 aa, Artificial Sequence
  PAS peptide
SSPSAPSPSSPASPSPSSPA

SEQ ID NO: 15 - protein, 24 aa, Artificial Sequence
  PAS peptide
AASPAAPSAPPAAASPAAPSAPPA

SEQ ID NO: 16 - protein, 20 aa, Artificial Sequence
  PAS peptide
ASAAAPAAASAAASAPSAAA